European Patent Specification EP 3 914 726 B1, published November 6, 2024. Title: Novel DNA repair protein and biomarker for  melanoma. Applicant: Council of Scientific and Industrial Research. The sequence listing filed with the application follows.

SEQUENCE LISTING (9 sequences)

SEQ ID NO: 1 - DNA, 3790 bp, Homo sapiens
agggaggggagggatggggggaaagcaagctggaggacaggtgagacagcaggacaggtgaggcgggccctgaggggggggcgggtgggagccaggtgaatgtacggctcttggcggccgagggggggcgggcggcaggaggaggcagagggcggcggaggaggagccccccagcagcgagcggcgagcaactgaccgcggccttctgaccaggaccggagcagggccccaagcccccgggcctggtgggggacgcgcttcttcccacactgtgagcctcagcagctccagccagcggacccgacggctgagaggagaagatggggagccccgaggatgacctgattgggattccattcccggaccacagcagtgagctcctgagctgcctcaatgagcagcgccagctgggccacctatgtgacctcaccatccggacgcagggccttgaataccgcacccacagggctgtgctagctgcctgtagccactacttcaagaagcttttcactgagggcggtggcggagctgtcatgggggccgggggtagcgggacggccactgggggagcaggggccggtgtgtgtgagctggactttgtagggccagaggcactaggcgccctccttgaatttgcctatacagccacactgaccaccagcagcgccaacatgccagctgtgctccaggctgcccgcctgctggagatcccgtgtgtcatcgctgcttgcatggagattctgcagggcagtgggctagaagctcccagcccggacgaggatgactgtgagcgagcccgccagtatctggaggcctttgccacagccacggcctctggagttcccaatggtgaagacagtcctccacaggtgcccctcccaccacctccgccaccgccacctcggcctgttgcccgccgcagccgcaagccccggaaagctttcctgcaaaccaagggggccagagcaaaccacctagtccctgaggtgcccacagtgcccgcccatcccttgacctatgaggaggaggaggtggcgggcagagtgggcagcagtgggggcagtgggccgggggacagctacagccctcccacaggaactgcctcccctcctgagggtccccagagctacgaaccctatgagggtgaggaagaagaagaggagctggtatatcccccagcctatgggctggcgcagggtggcgggcccccgctgtccccagaggagctgggctcagatgaggatgccatcgatcctgacctgatggcctacctaagctccctgcaccaggacaacctggcaccaggcctggacagccaagacaagctggtgcgcaaacgccgctcccagatgcctcaggagtgccctgtctgccacaagatcatccatggggcaggcaaactgcctcgccacatgaggacccacacaggcgagaagccctttgcctgcgaggtctgcggtgttcgattcaccaggaacgacaagctgaagatccacatgcggaagcacacgggagagcgcccctactcatgcccgcactgcccagcccgcttcctgcacagctacgacctcaagaaccacatgcacctgcacacaggggaccggccctatgagtgccacctgtgccacaaggctttcgccaaggaggaccacctgcagcgccacctcaaaggccagaactgcctggaggtgcgcacccgacggcgccgcaaggacgatgcaccaccccactacccaccaccctctaccgctgctgcatcccccgctggcctcgacctctccaatggccacctggacaccttccgcctctctctagctcgattctgggagcagtcagcccccactgggcccccggtctctaccccagggccccctgatgacgatgaggaggaaggggcacccaccacaccccaggctgaaggtgccatggagtcctcttaaagagggacgagggccagactgaagcagcacaaggccggggacacccatgccaagcagtgggagcacgcaggacagacacagcaggggtctggggcacggagccttgctggcatcagcatcagcccttcctcccagagccctcattccaattccaagctaagaaggtattggggcagaggctccccaaattggggtgatcccccaaggagtgatacatatattgtgtatatatttacagctgtattgtaaaagtggggtccctgtccccagctgctcctggggagtagaagcaataatgtatttctaatttgtgggtcccacttcggctatgcgggtttctagggggtgggggcttgggaccaaagccttgccccgcccctatgccccttgggggttttggctgtgtaagggggtgaaggactgcccctccctttcgagacccctccttcctggtttctgttcctttttcctggcagtgaattatgcaaagggggccggcaaaggaagggtaggtgggggaaagccaggtggaagcttgaaagactgggggactgggcctgtaaggaaggagccatcccagtccccctccgccctgctcccggcgctgagtcatggggtcgtggagaagggggcggggtggcctgattggctcgcctgcccctgggggcagtagaggggccccgcccagctaggggagccgctccgttccactcccctccctagccctccctccccacggccctgggcagggaatgtcttgttcccgccgctccctccccggggccagagggcagggcgggccgggcggcgtcctaccctcttctcctcctccccatctcctccccgcccaggtgcgagccggagccgccgccaccgctgccgcccctgactcacgccgcccccgggctggcgcagcgaagggtgtgggacagggtaaggggttggaagagccttgtggagagcgggcgagccggcgccatctggcggccatgctctgagtgggcgagcgccccccgcggccactggagcgagctgtcttcacgctcctcatccaccccagctggtgagcggcgcccccttgccaaggcagtgggcacagaacttctcgcttggccgcaggggaaggggctgcggacctgtgggaaagtgatccccttcccagatccttgccagccgggcttcctgtcaggcaggggagaataatccccactctgctcttaggattgaatccacccccattctgtacatagcctcttctgttggtcttgttgaaatctagtttcagatttttaactacccaattctgctgggggtgggggacacccccccttcctcgctgggtgctggaccccttttgcagcctgggctctgccttgcactatttccccttcctggcctgacggctcctccccctccttaaaaggggcaggttcaggggcccggtgctcttcctcccttccatgcacccccatgcccatttgcacagctgcccaggtacccctaacagtggggaggggtcacagggagggggtagcgggaccagtccctgttatctatttaaaaagtgatgatgtaatatattggggtggcggggagatcgggttgtcctgggcctcatcttagcatttcaggtgatggggggagcccagggctggggagacctggggcccagccccagaaagtggggacaatgtggcctcccttctccctactttcggctttcccagtcagtgccttagggggagaggcactccccccctcctattcccttccccccaccccaactcccccacctcgggtgtaagcgacaggaagaaataataataatttaagattcacaaaaaaaaaaa

SEQ ID NO: 2 - DNA, 1620 bp, Homo sapiens
atggggagccccgaggatgacctgattgggattccattcccggaccacagcagtgagctcctgagctgcctcaatgagcagcgccagctgggccacctatgtgacctcaccatccggacgcagggccttgaataccgcacccacagggctgtgctagctgcctgtagccactacttcaagaagcttttcactgagggcggtggcggagctgtcatgggggccgggggtagcgggacggccactgggggagcaggggccggtgtgtgtgagctggactttgtagggccagaggcactaggcgccctccttgaatttgcctatacagccacactgaccaccagcagcgccaacatgccagctgtgctccaggctgcccgcctgctggagatcccgtgtgtcatcgctgcttgcatggagattctgcagggcagtgggctagaagctcccagcccggacgaggatgactgtgagcgagcccgccagtatctggaggcctttgccacagccacggcctctggagttcccaatggtgaagacagtcctccacaggtgcccctcccaccacctccgccaccgccacctcggcctgttgcccgccgcagccgcaagccccggaaagctttcctgcaaaccaagggggccagagcaaaccacctagtccctgaggtgcccacagtgcccgcccatcccttgacctatgaggaggaggaggtggcgggcagagtgggcagcagtgggggcagtgggccgggggacagctacagccctcccacaggaactgcctcccctcctgagggtccccagagctacgaaccctatgagggtgaggaagaagaagaggagctggtatatcccccagcctatgggctggcgcagggtggcgggcccccgctgtccccagaggagctgggctcagatgaggatgccatcgatcctgacctgatggcctacctaagctccctgcaccaggacaacctggcaccaggcctggacagccaagacaagctggtgcgcaaacgccgctcccagatgcctcaggagtgccctgtctgccacaagatcatccatggggcaggcaaactgcctcgccacatgaggacccacacaggcgagaagccctttgcctgcgaggtctgcggtgttcgattcaccaggaacgacaagctgaagatccacatgcggaagcacacgggagagcgcccctactcatgcccgcactgcccagcccgcttcctgcacagctacgacctcaagaaccacatgcacctgcacacaggggaccggccctatgagtgccacctgtgccacaaggctttcgccaaggaggaccacctgcagcgccacctcaaaggccagaactgcctggaggtgcgcacccgacggcgccgcaaggacgatgcaccaccccactacccaccaccctctaccgctgctgcatcccccgctggcctcgacctctccaatggccacctggacaccttccgcctctctctagctcgattctgggagcagtcagcccccactgggcccccggtctctaccccagggccccctgatgacgatgaggaggaaggggcacccaccacaccccaggctgaaggtgccatggagtcctcttaa

SEQ ID NO: 3 - protein, 539 aa, Homo sapiens
MGSPEDDLIGIPFPDHSSELLSCLNEQRQLGHLCDLTIRTQGLEYRTHRAVLAACSHYFKKLFTEGGGGAVMGAGGSGTATGGAGAGVCELDFVGPEALGALLEFAYTATLTTSSANMPAVLQAARLLEIPCVIAACMEILQGSGLEAPSPDEDDCERARQYLEAFATATASGVPNGEDSPPQVPLPPPPPPPPRPVARRSRKPRKAFLQTKGARANHLVPEVPTVPAHPLTYEEEEVAGRVGSSGGSGPGDSYSPPTGTASPPEGPQSYEPYEGEEEEEELVYPPAYGLAQGGGPPLSPEELGSDEDAIDPDLMAYLSSLHQDNLAPGLDSQDKLVRKRRSQMPQECPVCHKIIHGAGKLPRHMRTHTGEKPFACEVCGVRFTRNDKLKIHMRKHTGERPYSCPHCPARFLHSYDLKNHMHLHTGDRPYECHLCHKAFAKEDHLQRHLKGQNCLEVRTRRRRKDDAPPHYPPPSTAAASPAGLDLSNGHLDTFRLSLARFWEQSAPTGPPVSTPGPPDDDEEEGAPTTPQAEGAMESS

SEQ ID NO: 4 - DNA, 20 bp, Artificial Sequence
  vGAF fwd primer
cggtgttcgattcaccagga

SEQ ID NO: 5 - DNA, 20 bp, Artificial Sequence
  vGAF rev primer
gcaggtgcatgtggttcttg

SEQ ID NO: 6 - DNA, 20 bp, Artificial Sequence
  hist1H3A fwd primer
ggctcgcactaagcaaactg

SEQ ID NO: 7 - DNA, 20 bp, Artificial Sequence
  Hist1H3A rev primer
ctgccttagtggccaactgt

SEQ ID NO: 8 - DNA, 20 bp, Artificial Sequence
  Col1A1 fwd primer
agtggtttggatggtgccaa

SEQ ID NO: 9 - DNA, 20 bp, Artificial Sequence
  Col1A1 rev primer
gcaccatcatttccacgagc